European Patent Specification EP 3 248 614 B1, published May 21, 2025. Title: METHODS AND KITS FOR TOPICAL APPLICATION, REMOVAL, AND INACTIVATION OF THERAPEUTIC OR COSMETIC TOXIN COMPOSITIONS. Applicant: REVANCE THERAPEUTICS, INC. Application EP 11855190.2. The sequence listing filed with the application follows.

SEQUENCE LISTING (6 sequences)

SEQ ID NO: 1 - protein, 45 aa, Artificial Sequence
  Description of Artificial Sequence: Synthetic polypeptide
  misc_feature (1)..(20): This region may encompass 0 to 20 residues, wherein some residues may be absent
  misc_feature (21)..(45): This region may encompass 5, 7, 9, 11, 13, 15, 17, 19, 21, 23 or 25 residues, wherein some residues may be absent
GGGGGGGGGGGGGGGGGGGGRRRRRRRRRRRRRRRRRRRRRRRRR

SEQ ID NO: 2 - protein, 51 aa, Human immunodeficiency virus
  misc_feature (1)..(20): This region may encompass 0 to 20 residues, wherein some residues may be absent
  misc_feature (32)..(51): This region may encompass 0 to 20 residues, wherein some residues may be absent
GGGGGGGGGGGGGGGGGGGGRGRDDRRQRRRGGGGGGGGGGGGGGGGGGGG

SEQ ID NO: 3 - protein, 51 aa, Human immunodeficiency virus
  misc_feature (1)..(20): This region may encompass 0 to 20 residues, wherein some residues may be absent
  misc_feature (32)..(51): This region may encompass 0 to 20 residues, wherein some residues may be absent
GGGGGGGGGGGGGGGGGGGGYGRKKRRQRRRGGGGGGGGGGGGGGGGGGGG

SEQ ID NO: 4 - protein, 49 aa, Human immunodeficiency virus
  misc_feature (1)..(20): This region may encompass 0 to 20 residues, wherein some residues may be absent
  misc_feature (30)..(49): This region may encompass 0 to 20 residues, wherein some residues may be absent
GGGGGGGGGGGGGGGGGGGGRKKRRQRRRGGGGGGGGGGGGGGGGGGGG

SEQ ID NO: 5 - protein, 35 aa, Artificial Sequence
  Description of Artificial Sequence: Synthetic polypeptide
RKKRRQRRRGKKKKKKKKKKKKKKKGRKKRRQRRR

SEQ ID NO: 6 - protein, 10 aa, Artificial Sequence
  Description of Artificial Sequence: Synthetic peptide
GGGRRRRRRR